European Patent Specification EP 3 946 435 B1, published December 27, 2023. Title: ENHANCEMENT OF CYTOLYTIC T-CELL ACTIVITY BY INHIBITING EBAG9. Applicant: Max-Delbrück-Centrum für Molekulare Medizin in der Helmholtz-Gemeinschaft. The sequence listing filed with the application follows.

SEQUENCE LISTING (62 sequences)

SEQ ID NO: 1 - DNA, 21 bp, Homo sapiens
aaataaccgaaactgggtgat

SEQ ID NO: 2 - DNA, 21 bp, Homo sapiens
ttaaataaccgaaactgggtg

SEQ ID NO: 3 - DNA, 2383 bp, Homo sapiens
aggcgtgcagcattcgccatgctccgctcacgcgtgggagactgggctgtggggtaccggcccggaaagcacgcagcctccaaagccgccttcctcagggaaatttgcgtgaccttactgccctccgtctacaggccttgtacctctccaggccgatttttccacaatttaaatctcagttcacctggtatccagctccagcaacttagagcgtttcacgtcacgccgggcgccaggcgtcggcttgtataacctgaaaacgctcctgtttttctcatctgtgcagtgggttttgattcccaccatggccatcacccagtttcggttatttaaattttgtacctgcctagcaacagtattctcattcctaaagagattaatatgcagatctggcagaggacggaaattaagtggagaccaaataactttgccaactacagttgattattcatcagttcctaagcagacagatgttgaagagtggacttcctgggatgaagatgcacccaccagtgtaaagatcgaaggagggaatgggaatgtggcaacacaacaaaattctttggaacaactggaacctgactattttaaggacatgacaccaactattaggaaaactcagaaaattgttattaagaagagagaaccattgaattttggcatcccagatgggagcacaggtttctctagtagattagcagctacacaagatctgccttttattcatcagtcttctgaattaggtgacttagatacctggcaggaaaataccaatgcatgggaagaagaagaagatgcagcctggcaagcagaagaagttctgagacagcagaaactagcagacagagaaaagagagcagccgaacaacaaaggaagaaaatggaaaaggaagcacaacggctaatgaagaaggaacaaaacaaaattggtgtgaaactttcataacacatgttcaaattttatcatgccagtaggagaaatctcagctccacaacccaagcaacatttgtatggatttaagagtattttaagaagacatactgcttgattttaatacattgatcaggccatccaggacaccacgattctcccaaagtaccttgaactcttagtgattgagactcaaaaaaacaaaaaagacttgagacaatgttttcttcaacatgctccaaatataagacatttgtttgctgtacagaaagtatcacaaatggaatatatcagtacctctcaagctagtgtttctagctaaataaatgggtgtatataattttatggtggaaaagaactgtactgtctgttatgatttccttcaatgtgcataatgataaaataaataattttaatattcttttgtttccatggttacctgacctaaattagataaattgtagggctttagctttcttatttttgtcaaaagttggtgttgacatacattccctctaatttgaactggtattgtttacgtttgatacaacattaaggaatttgatgattttcatttcatgaaaatgacattaaatgcaataattttacttatcataaacattttgtacatcattattttcttttggattagtgttgtcatacatgtaatttatatcacatgtataaacattgaaaatcaactaaaatgacatttgttctacattataacttgtgagtttcaagaactagtattagtagttttttcctttcattatagattgtaagatgttgtggtatctttgagtgccttagttcttccttcctcccaaaagccattaatttacaaatgcttaaagccatcaggtcaaatatttcaaagcctttagatgatttctgtactagctttagatgtctgacgttatgtaggttacctgtgttcttggctaggaaaacattattgattcattaaatcataaaggtgggaataataatcttttatttatgatgttgattggctccaaaatagtcttaaggaaataaatactgggtctgtaggggaaaagtagacttcatagtttaaaatcccattaaccttttcaccgcagttgaaatgcatccagcctgattttcctatcattttggaatttttaaggatttttactttcttaagttactgcctagaatcaacattcggtgagattttgaaatgtcatagatactgtacaggccaaaccttactaatttattttacttaaagtgatattttatagaaaaatcataagttatacaatgagaaccctttaagcccttagcctaagctttcagactaaatgtgattatagaataagatgaaagttaactttggtacagagctttttatagccccaaattatatttccagttattatattcattagaatttctgctaataaactcccaacttaaatagaa

SEQ ID NO: 4 - DNA, 2328 bp, Homo sapiens
gcgggtttcccgatgaaggggcggccatggcagctgcgcagaggcaacgcaggctgctacggagcgcgcgcccggctttgaatgagcggggctgggagtgagcgggcggagcgcgagctcgaggaagagacaggcagcgcgcgtgagcgcgccttgtgtgcgcgcgcggcccgcggcagctcggagcctccgccgggcgggcggggagggggaggggcaggttttgattcccaccatggccatcacccagtttcggttatttaaattttgtacctgcctagcaacagtattctcattcctaaagagattaatatgcagatctggcagaggacggaaattaagtggagaccaaataactttgccaactacagttgattattcatcagttcctaagcagacagatgttgaagagtggacttcctgggatgaagatgcacccaccagtgtaaagatcgaaggagggaatgggaatgtggcaacacaacaaaattctttggaacaactggaacctgactattttaaggacatgacaccaactattaggaaaactcagaaaattgttattaagaagagagaaccattgaattttggcatcccagatgggagcacaggtttctctagtagattagcagctacacaagatctgccttttattcatcagtcttctgaattaggtgacttagatacctggcaggaaaataccaatgcatgggaagaagaagaagatgcagcctggcaagcagaagaagttctgagacagcagaaactagcagacagagaaaagagagcagccgaacaacaaaggaagaaaatggaaaaggaagcacaacggctaatgaagaaggaacaaaacaaaattggtgtgaaactttcataacacatgttcaaattttatcatgccagtaggagaaatctcagctccacaacccaagcaacatttgtatggatttaagagtattttaagaagacatactgcttgattttaatacattgatcaggccatccaggacaccacgattctcccaaagtaccttgaactcttagtgattgagactcaaaaaaacaaaaaagacttgagacaatgttttcttcaacatgctccaaatataagacatttgtttgctgtacagaaagtatcacaaatggaatatatcagtacctctcaagctagtgtttctagctaaataaatgggtgtatataattttatggtggaaaagaactgtactgtctgttatgatttccttcaatgtgcataatgataaaataaataattttaatattcttttgtttccatggttacctgacctaaattagataaattgtagggctttagctttcttatttttgtcaaaagttggtgttgacatacattccctctaatttgaactggtattgtttacgtttgatacaacattaaggaatttgatgattttcatttcatgaaaatgacattaaatgcaataattttacttatcataaacattttgtacatcattattttcttttggattagtgttgtcatacatgtaatttatatcacatgtataaacattgaaaatcaactaaaatgacatttgttctacattataacttgtgagtttcaagaactagtattagtagttttttcctttcattatagattgtaagatgttgtggtatctttgagtgccttagttcttccttcctcccaaaagccattaatttacaaatgcttaaagccatcaggtcaaatatttcaaagcctttagatgatttctgtactagctttagatgtctgacgttatgtaggttacctgtgttcttggctaggaaaacattattgattcattaaatcataaaggtgggaataataatcttttatttatgatgttgattggctccaaaatagtcttaaggaaataaatactgggtctgtaggggaaaagtagacttcatagtttaaaatcccattaaccttttcaccgcagttgaaatgcatccagcctgattttcctatcattttggaatttttaaggatttttactttcttaagttactgcctagaatcaacattcggtgagattttgaaatgtcatagatactgtacaggccaaaccttactaatttattttacttaaagtgatattttatagaaaaatcataagttatacaatgagaaccctttaagcccttagcctaagctttcagactaaatgtgattatagaataagatgaaagttaactttggtacagagctttttatagccccaaattatatttccagttattatattcattagaatttctgctaataaactcccaacttaaatagaaaaaaaaaaaaaaaa

SEQ ID NO: 5 - DNA, 2208 bp, Homo sapiens
atggcacagaatgttcgattttactaccagctctcacactccgcttctgtttccccttctcttacgggccgctgctcaaacctttatttatcaaatttaagttttgattcccaccatggccatcacccagtttcggttatttaaattttgtacctgcctagcaacagtattctcattcctaaagagattaatatgcagatctggcagaggacggaaattaagtggagaccaaataactttgccaactacagttgattattcatcagttcctaagcagacagatgttgaagagtggacttcctgggatgaagatgcacccaccagtgtaaagatcgaaggagggaatgggaatgtggcaacacaacaaaattctttggaacaactggaacctgactattttaaggacatgacaccaactattaggaaaactcagaaaattgttattaagaagagagaaccattgaattttggcatcccagatgggagcacaggtttctctagtagattagcagctacacaagatctgccttttattcatcagtcttctgaattaggtgacttagatacctggcaggaaaataccaatgcatgggaagaagaagaagatgcagcctggcaagcagaagaagttctgagacagcagaaactagcagacagagaaaagagagcagccgaacaacaaaggaagaaaatggaaaaggaagcacaacggctaatgaagaaggaacaaaacaaaattggtgtgaaactttcataacacatgttcaaattttatcatgccagtaggagaaatctcagctccacaacccaagcaacatttgtatggatttaagagtattttaagaagacatactgcttgattttaatacattgatcaggccatccaggacaccacgattctcccaaagtaccttgaactcttagtgattgagactcaaaaaaacaaaaaagacttgagacaatgttttcttcaacatgctccaaatataagacatttgtttgctgtacagaaagtatcacaaatggaatatatcagtacctctcaagctagtgtttctagctaaataaatgggtgtatataattttatggtggaaaagaactgtactgtctgttatgatttccttcaatgtgcataatgataaaataaataattttaatattcttttgtttccatggttacctgacctaaattagataaattgtagggctttagctttcttatttttgtcaaaagttggtgttgacatacattccctctaatttgaactggtattgtttacgtttgatacaacattaaggaatttgatgattttcatttcatgaaaatgacattaaatgcaataattttacttatcataaacattttgtacatcattattttcttttggattagtgttgtcatacatgtaatttatatcacatgtataaacattgaaaatcaactaaaatgacatttgttctacattataacttgtgagtttcaagaactagtattagtagttttttcctttcattatagattgtaagatgttgtggtatctttgagtgccttagttcttccttcctcccaaaagccattaatttacaaatgcttaaagccatcaggtcaaatatttcaaagcctttagatgatttctgtactagctttagatgtctgacgttatgtaggttacctgtgttcttggctaggaaaacattattgattcattaaatcataaaggtgggaataataatcttttatttatgatgttgattggctccaaaatagtcttaaggaaataaatactgggtctgtaggggaaaagtagacttcatagtttaaaatcccattaaccttttcaccgcagttgaaatgcatccagcctgattttcctatcattttggaatttttaaggatttttactttcttaagttactgcctagaatcaacattcggtgagattttgaaatgtcatagatactgtacaggccaaaccttactaatttattttacttaaagtgatattttatagaaaaatcataagttatacaatgagaaccctttaagcccttagcctaagctttcagactaaatgtgattatagaataagatgaaagttaactttggtacagagctttttatagccccaaattatatttccagttattatattcattagaatttctgctaataaactcccaacttaaatagaaaaaaaaaaaaaaaa

SEQ ID NO: 6 - DNA, 1844 bp, Homo sapiens
tgcgactgggagcgggacccaggcgtgcagcattcgccatgctccgctcacgcgtgggagactgggctgtggggtaccggcccggaaagcacgcagcctccaaagccgccttcctcagggaaatttgcgtgaccttactgccctccgtctacaggccttgtacctctccaggccgatttttccacaatttaaatctcagttcacctggtatccagctccagcaacttagagcgtttcacgtcacgccgggcgccaggcgtcggcttgtataacctgaaaacgctcctgtttttctcatctgtgcagtgggtatgatttttttttcatcaacaaatttcacgtgggtaatctgaaatgaaaccacttaagttatgaaactctttccttttgagttattctggagaccttactccgccttcggaaccgccccagtggtgtcacatacttgagggcctgactctcggttgccagacatggcacagaatgttcgattttactaccagctctcacactccgcttctgtttccccttctcttacgggccgctgctcaaacctttatttatcaaatttaagtgagttcaggttttgattcccaccatggccatcacccagtttcggttatttaaattttgtacctgcctagcaacagtattctcattcctaaagagattaatatgcagatctggcagaggacggaaattaagtggagaccaaataactttgccaactacagttgattattcatcagttcctaagcagacagatgttgaagagtggacttcctgggatgaagatgcacccaccagtgtaaagatcgaaggagggaatgggaatgtggcaacacaacaaaattctttggaacaactggaacctgactattttaaggacatgacaccaactattaggaaaactcagaaaattgttattaagaagagagaaccattgaattttggcatcccagatgggagcacaggtttctctagtagattagcagctacacaagatctgccttttattcatcagtcttctgaattaggtgacttagatacctggcaggaaaataccaatgcatgggaagaagaagaagatgcagcctggcaagcagaagaagttctgagacagcagaaactagcagacagagaaaagagagcagccgaacaacaaaggaagaaaatggaaaaggaagcacaacggctaatgaagaaggaacaaaacaaaattggtgtgaaactttcataacacatgttcaaattttatcatgccagtaggagaaatctcagctccacaacccaagcaacatttgtatggatttaagagtattttaagaagacatactgcttgattttaatacattgatcaggccatccaggacaccacgattctcccaaagtaccttgaactcttagtgattgagactcaaaaaaacaaaaaagacttgagacaatgttttcttcaacatgctccaaatataagacatttgtttgctgtacagaaagtatcacaaatggaatatatcagtacctctcaagctagtgtttctagctaaataaatgggtgtatataattttatggtggaaaagaactgtactgtctgttatgatttccttcaatgtgcataatgataaaataaataattttaatattcttttgtttccatggttacctgacctaaattagataaattgtagggctttagctttcttatttttgtcaaaagttggtgttgacatacattccctctaatttgaactggtattgtttacgtttgatacaacattaaggaatttgatgattttcatttcatgaaaatgacattaaatgcaataattttacttatcataaa

SEQ ID NO: 7 - protein, 8 aa, Artificial Sequence
  CDR
GFTFSTSG

SEQ ID NO: 8 - protein, 8 aa, Artificial Sequence
  CDR
ISSSSGFV

SEQ ID NO: 9 - protein, 7 aa, Artificial Sequence
  CDR
ARSEAAF

SEQ ID NO: 10 - protein, 11 aa, Artificial Sequence
  CDR
KSRLSRMGITP

SEQ ID NO: 11 - protein, 9 aa, Artificial Sequence
  CDR
AQFLEYPPT

SEQ ID NO: 12 - protein, 113 aa, Artificial Sequence
  VH
EVQLVESGGGLVQPGGSLRLSCAASGFTFSTSGMNWFRQAPGKGLEWVSYISSSSGFVYADSVKGRFTISRDNAQNSLYLQMNSLRAEDTAVYYCARSEAAFWGQGTLVTVSS

SEQ ID NO: 13 - protein, 113 aa, Artificial Sequence
  VH
EVQLVESGGGLVQPGKSLKLSCSASGFTFSTSGMHWFRQAPGKGLDWVAYISSSSGFVYADAVKGRFTISRDNAQNTLYLQLNSLKSEDTAIYYCARSEAAFWGQGTLVTVSS

SEQ ID NO: 14 - protein, 112 aa, Artificial Sequence
  VL
DIVLTQSPRSLPVTPGEPASISCRSSKSRLSRMGITPLNWYLQKPGQSPQLLIYRMSNRASGVPDRFSGSGSGTDFTLKISKVETEDVGVYYCAQFLEYPPTFGSGTKLEIK

SEQ ID NO: 15 - protein, 112 aa, Artificial Sequence
  VL
DIVLTQAPRSVSVTPGESASISCRSNKSRLSRMGITPLNWYLQKPGKSPQLLIYRMSNLASGVPDRFSGSGSETDFTLKISKVETEDVGVYYCAQFLEYPPTFGSGTKLEIK

SEQ ID NO: 16 - protein, 8 aa, Artificial Sequence
  CDR
GFTFSRYW

SEQ ID NO: 17 - protein, 8 aa, Artificial Sequence
  CDR
INPSSSTI

SEQ ID NO: 18 - protein, 13 aa, Artificial Sequence
  CDR
ASLYYDYGDAYDY

SEQ ID NO: 19 - protein, 6 aa, Artificial Sequence
  CDR
QSVESN

SEQ ID NO: 20 - protein, 9 aa, Artificial Sequence
  CDR
QQYNNYPLT

SEQ ID NO: 21 - protein, 5 aa, Artificial Sequence
  CDR
RYWFS

SEQ ID NO: 22 - protein, 18 aa, Artificial Sequence
  CDR
EINPSSSTINYAPSLKDK

SEQ ID NO: 23 - protein, 13 aa, Artificial Sequence
  CDR
SLYYDYGDAYDYW

SEQ ID NO: 24 - protein, 11 aa, Artificial Sequence
  CDR
KASQSVESNVA

SEQ ID NO: 25 - protein, 7 aa, Artificial Sequence
  CDR
SASLRFS

SEQ ID NO: 26 - protein, 11 aa, Artificial Sequence
  CDR
QQYNNYPLTFG

SEQ ID NO: 27 - protein, 120 aa, Artificial Sequence
  VH
EVQLVESGGGLVQPGGSLRLSCAASGFTFSRYWFSWVRQAPGKGLVWVGEINPSSSTINYAPSLKDKFTISRDNAKNTLYLQMNSLRAEDTAVYYCASLYYDYGDAYDYWGQGTLVTVSS

SEQ ID NO: 28 - protein, 107 aa, Artificial Sequence
  VL
EIVMTQSPATLSVSPGERATLSCKASQSVESNVAWYQQKPGQAPRALIYSASLRFSGIPARFSGSGSGTEFTLTISSLQSEDFAVYYCQQYNNYPLTFGAGTKLELK

SEQ ID NO: 29 - protein, 18 aa, Artificial Sequence
  linker
GSTSGSGKPGSGEGSTKG

SEQ ID NO: 30 - protein, 17 aa, Artificial Sequence
  linker
SSGGGGSGGGGSGGGGS

SEQ ID NO: 31 - protein, 237 aa, Artificial Sequence
  spacer
PAEPKSPDKTHTCPPCPAPPVAGPSVFLFPPKPKDTLMIARTPEVTCVVVDVSHEDPEVKFNWYVDGVEVHNAKTKPREEQYNSTYRVVSVLTVLHQDWLNGKEYKCKVSNKALPAPIEKTISKAKGQPREPQVYTLPPSRDELTKNQVSLTCLVKGFYPSDIAVEWESNGQPENNYKTTPPVLDSDGSFFLYSKLTVDKSRWQQGNVFSCSVMHEALHNHYTQKSLSLSPGKKDPK

SEQ ID NO: 32 - protein, 235 aa, Artificial Sequence
  spacer
PAEPKSPDKTHTCPPCPAPPVAGPSVFLFPPKPKDTLMIARTPEVTCVVVDVSHEDPEVKFNWYVDGVEVHNAKTKPREEQYNSTYRVVSVLTVLHQDWLNGKEYKCKVSNKALPAPIEKTISKAKGQPREPQVYTLPPSRDELTKNQVSLTCLVKGFYPSDIAVEWESNGQPENNYKTTPPVLDSDGSFFLYSKLTVDKSRWQQGNVFSCSVMHEALHNHYTQKSLSSLSPGKK

SEQ ID NO: 33 - protein, 229 aa, Artificial Sequence
  spacer
ESKYGPPCPPCPAPEFEGGPSVFLFPPKPKDTLMISRTPEVTCVVVDVSQEDPEVQFNWYVDGVEVHNAKTKPREEQFNSTYRVVSVLTVLHQDWLNGKEYKCKVSNKGLPSSIEKTISKAKGQPREPQVYTLPPSQEEMTKNQVSLTCLVKGFYPSDIAVEWESNGQPENNYKTTPPVLDSDGSFFLYSRLTVDKSRWQEGNVFSCSVMHEALHNHYTQKSLSLSLGK

SEQ ID NO: 34 - protein, 119 aa, Artificial Sequence
  spacer
ESKYGPPCPPCPGQPREPQVYTLPPSQEEMTKNQVSLTCLVKGFYPSDIAVEWESNGQPENNYKTTPPVLDSDGSFFLYSRLTVDKSRWQEGNVFSCSVMHEALHNHYTQKSLSLSLGK

SEQ ID NO: 35 - protein, 12 aa, Artificial Sequence
  spacer
ESKYGPPCPPCP

SEQ ID NO: 36 - protein, 24 aa, Artificial Sequence
  transmembrane
IYIWAPLAGTCGVLLLSLVITLYC

SEQ ID NO: 37 - protein, 27 aa, Artificial Sequence
  transmembrane
FWVLVVVGGVLACYSLLVTVAFIIFWV

SEQ ID NO: 38 - protein, 42 aa, Artificial Sequence
  Co-stimulatory domain
KRGRKKLLYIFKQPFMRPVQTTQEEDGCSCRFPEEEEGGCEL

SEQ ID NO: 39 - protein, 42 aa, Artificial Sequence
  Co-stimulatory domain
RSKRSRLLHSDYMNMTPRRPGPTRKHYQPYAPPRDFAAYRSL

SEQ ID NO: 40 - protein, 113 aa, Artificial Sequence
  Activation domain
LRVKFSRSADAPAYQQGQNQLYNELNLGRREEYDVLDKRRGRDPEMGGKPRRKNPQEGLYNELQKDKMAEAYSEIGMKGERRRGKGHDGLYQGLSTATKDTYDALHMQALPPR

SEQ ID NO: 41 - protein, 21 aa, Artificial Sequence
  leader
MDFQVQIFSFLLISASVIMSR

SEQ ID NO: 42 - DNA, 63 bp, Artificial Sequence
  leader
atggatttccaggtgcagatcttcagcttcctgctgatctccgccagcgtgatcatgagccgc

SEQ ID NO: 43 - DNA, 54 bp, Artificial Sequence
  linker
ggcagcacaagcggctctggcaaacctggatctggcgagggcagcaccaagggc

SEQ ID NO: 44 - DNA, 54 bp, Artificial Sequence
  linker
ggcagcaccagcggctccggcaagcctggctctggcgagggcagcacaaaggga

SEQ ID NO: 45 - DNA, 711 bp, Artificial Sequence
  spacer
cccgccgagcccaagagccccgacaagacccatacctgccctccatgtcctgcccctccagtggctggccctagcgtgttcctgttccccccaaagcccaaggacaccctgatgatcgcccggacccctgaagtgacctgcgtggtggtggatgtgtcccacgaggatcccgaagtgaagttcaattggtacgtggacggcgtggaagtgcacaacgccaagaccaagcccagagaggaacagtacaacagcacctaccgggtggtgtctgtgctgaccgtgctgcatcaggactggctgaacggcaaagagtacaagtgcaaggtgtccaacaaggccctgcctgcccccatcgagaaaaccatctccaaggccaagggacagccccgcgagccccaggtgtacacactgcctccaagcagggacgagctgaccaagaaccaggtcagcctgacctgcctggtcaaaggcttctatcccagcgacatcgccgtggagtgggagagcaatgggcagccggagaacaactacaagaccacgcctcccgtgctggactccgacggctccttcttcctctacagcaagctcaccgtggacaagagcaggtggcagcaggggaacgtcttctcatgctccgtgatgcatgaggctctgcacaaccactacacgcagaagagcctctccctgtctccgggtaaaaaagatcccaaa

SEQ ID NO: 46 - DNA, 711 bp, Artificial Sequence
  spacer
cctgccgagcctaagagccccgacaagacccacacctgtcccccttgtcctgcccctccagtggctggccctagcgtgttcctgttccccccaaagcccaaggataccctgatgatcgcccggacccccgaagtcacatgcgtggtggtggacgtgagccacgaagaccctgaggtcaagttcaactggtacgtggacggcgtggaggtgcataatgccaagacaaagccgcgggaggagcagtacaacagcacgtaccgtgtggtcagcgtcctcaccgtcctgcaccaggactggctgaatggcaaggagtacaagtgcaaggtctccaacaaagccctcccagcccccatcgagaaaaccatctccaaagccaaagggcagccccgagaaccacaggtgtacaccctgcccccatcccgggatgagctgaccaagaaccaggtcagcctgacctgcctggtcaaaggcttctatcccagcgacatcgccgtggagtgggagagcaatgggcagccggagaacaactacaagaccacgcctcccgtgctggactccgacggctccttcttcctctacagcaagctcaccgtggacaagagcaggtggcagcaggggaacgtcttctcatgctccgtgatgcatgaggctctgcacaaccactacacgcagaagagcctctccctgtctccgggtaaaaaagatcccaaa

SEQ ID NO: 47 - DNA, 265 bp, Artificial Sequence
  spacer
ccaggtgtccctgacctgcctcgtgaagggcttctacccctccgatatcgccgtggaatgggagagcaatggccagcccgagaacaactacaagaccaccccccctgtgctggacagcgacggctcattcttcctgtacagcaagctgacagtggacaagagccggtggcagcagggcaacgtgttcagctgcagcgtgatgcacgaggctctgcacaaccactacacccagaagtccctgagcagcctgagcccaggcaagaag

SEQ ID NO: 48 - DNA, 440 bp, Artificial Sequence
  spacer
cctgccgagcctaagagccccgacaagacccacacctgtcccccttgtcctgcccctccagtggctggccctagcgtgttcctgttccccccaaagcccaaggataccctgatgatcgcccggacccccgaagtcacatgcgtggtggtggacgtgagccacgaagaccctgaggtcaagttcaactggtacgtggacggcgtggaggtgcataatgccaagacaaagccgcgggaggagcagtacaacagcacgtaccgtgtggtcagcgtcctcaccgtcctgcaccaggactggctgaatggcaaggagtacaagtgcaaggtctccaacaaagccctcccagcccccatcgagaaaaccatctccaaagccaaagggcagccccgagaaccacaggtgtacaccctgcccccatcccgggatgagctgaccaagaa

SEQ ID NO: 49 - DNA, 72 bp, Artificial Sequence
  transmembrane domain
atctacatctgggcccctctggccggcacctgtggcgtgctgctgctgtctctcgtgatcacactgtactgc

SEQ ID NO: 50 - DNA, 81 bp, Artificial Sequence
  transmembrane domain
ttttgggtgctggtggtggttggtggagtcctggcttgctatagcttgctagtaacagtggcctttattattttctgggtg

SEQ ID NO: 51 - DNA, 126 bp, Artificial Sequence
  Co-stimulatory domain
aagcggggcagaaagaagctgctgtacatcttcaagcagcccttcatgcggcccgtgcagaccacccaggaagaggacggctgctcctgcagattccccgaggaagaagaaggcggctgcgagctg

SEQ ID NO: 52 - DNA, 126 bp, Artificial Sequence
  Co-stimulatory domain
aggagtaagaggagcaggctcctgcacagtgactacatgaacatgactccccgccgccccgggcccacccgcaagcattaccagccctatgccccaccacgcgacttcgcagcctatcgctccctg

SEQ ID NO: 53 - DNA, 342 bp, Artificial Sequence
  Activation domain
ctgcgcgtgaagttttctagaagcgccgacgcccctgcctaccagcagggccagaaccagctgtacaacgagctgaacctgggcagacgggaagagtacgacgtgctggataagcggagaggccgggaccctgagatgggcggcaagcctagaagaaagaacccccaggaaggcctgtataacgaactgcagaaagacaagatggccgaggcctacagcgagatcggaatgaagggcgagcggagaagaggcaagggccacgatggactgtaccagggcctgagcaccgccaccaaggacacctatgacgccctgcacatgcaggctctgccccccagataa

SEQ ID NO: 54 - DNA, 339 bp, Artificial Sequence
  Activation domain
agagtgaagttcagcaggagcgcagacgcccccgcgtaccagcagggccagaaccagctctataacgagctcaatctaggacgaagagaggagtacgatgttttggacaagagacgtggccgggaccctgagatggggggaaagccgagaaggaagaaccctcaggaaggcctgtacaatgaactgcagaaagataagatggcggaggcctacagtgagattgggatgaaaggcgagcgccggaggggcaaggggcacgatggcctttaccagggtctcagtacagccaccaaggacacctacgacgcccttcacatgcaggccctgccccctcgctga

SEQ ID NO: 55 - DNA, 21 bp, Homo sapiens
taaataaccgaaactgggtga

SEQ ID NO: 56 - DNA, 21 bp, Homo sapiens
taggaatgagaatactgttgc

SEQ ID NO: 57 - DNA, 21 bp, Homo sapiens
cttaatttccgtcctctgcca

SEQ ID NO: 58 - DNA, 21 bp, Homo sapiens
tttggtctccacttaatttcc

SEQ ID NO: 59 - DNA, 21 bp, Homo sapiens
ttcaacatctgtctgcttagg

SEQ ID NO: 60 - DNA, 21 bp, Homo sapiens
aagtccactcttcaacatctg

SEQ ID NO: 61 - DNA, 21 bp, Homo sapiens
atcccaggaagtccactcttc

SEQ ID NO: 62 - DNA, 21 bp, Homo sapiens
tactagagaaacctgtgctcc